European Patent Application EP 4 768 592 A1, published July 1, 2026. Title: RAC1 5'UTR-derived nucleic acid sequences for enhancing protein expression. Applicant: 단국대학교 산학협력단. Application EP. The sequence listing filed with the application follows.

SEQUENCE LISTING (69 sequences)

SEQ ID NO: 1 - DNA, 279 bp, synthetic construct
  source 1..279: mol_type = other DNA
gaggggctgggagccgcggcggggcggtgcgagggcgggccggggccggttccgcgcgcagggattttaaatgtcccgctctgagccgggcgcaggagcagccggcgcggccgccagcgcggtgtagggggcaggcgcggatcccgccaccgccgcgcgctcggcccgccgactcccggcgccgccgccgccactgccgtcgccgccgccgcctgccgggactggagcgcgccgtccgccgcggacaagaccctggcctcaggccggagcagccccatc

SEQ ID NO: 2 - DNA, 511 bp, synthetic construct
  source 1..511: mol_type = other DNA
gacgtcggcccgccggcgccccaccagctccgcgcgggcccgggttggccaccgccgggcccccgcccctcccccggcggtgtcccggccggaaccgatcgtggctggtttgagctggtgcgtctccatggcgacccgccggtgctataagtagggagcggcgtgccgtggggctttgtcagtccctcctgtagccgccgccgccgccgcccgccgcccctctgccagcagctccggcgccacctcgggccggcgtctccggcgggcgggagccaggcgctgacgggcgcggcgggggcggccgagcgctcctgcggctgcgactcaggctccggcgtctgcgcttccccatggggctggcctgcggcgcctgggcgctctgagattgtcactgctgttccaagggcacacgcagagggatttggaattcctggagagttgcctttgtgagaagctggaaatatttctttcaattccatctcttagttttccataggaacatcaagaaatc

SEQ ID NO: 3 - DNA, 197 bp, synthetic construct
  source 1..197: mol_type = other DNA
agttttcctcagctttgggtggtggccgctgccgggcatcggcttccagtccgcggagggcgaggcggcgtggacagcggccccggcacccagcgccccgccgcccgcaagccgcgcgcccgtccgccgcgccccgagcccgccgcttcctatctcagcgccctgccgccgccgccgcggcccagcgagcggccctg

SEQ ID NO: 4 - DNA, 47 bp, synthetic construct
  source 1..47: mol_type = other DNA
acatttgcttctgacacaactgtgttcactagcaacctcaaacagac

SEQ ID NO: 5 - DNA, 50 bp, synthetic construct
  source 1..50: mol_type = other DNA
gaataaactagtatctctggtccccacagactcagagagaacccgccacc

SEQ ID NO: 6 - DNA, 153 bp, synthetic construct
  source 1..153: mol_type = other DNA
agagactctccgaggcggcggcagagacagaagagcggggtcggggccggctgaccaggaacctgggcgagcagcggcgggggcccgagggattctgaaggaagatttccattaggtaatttgtttaatcagtgcaagcgaaattaagggaaa

SEQ ID NO: 7 - DNA, 233 bp, synthetic construct
  source 1..233: mol_type = other DNA
gcctcggccaataagcgccgccctctcgcccccgtgttactgggtagaagaaaacaaaaacaaacagagcgagaagggccagagactctccgaggcggcggcagagacagaagagcggggtcggggccggctgaccaggaacctgggcgagcagcggcgggggcccgagggattctgaaggaagatttccattaggtaatttgtttaatcagtgcaagcgaaattaagggaaa

SEQ ID NO: 8 - DNA, 50 bp, synthetic construct
  source 1..50: mol_type = other DNA
tagatccttttaaattaaaaatgaagttttaaatcaatctaaagtatata

SEQ ID NO: 9 - DNA, 29 bp, synthetic construct
  source 1..29: mol_type = other DNA
gggaagcttgaggggctgggagccgcggc

SEQ ID NO: 10 - DNA, 29 bp, synthetic construct
  source 1..29: mol_type = other DNA
cccccatgggatggggctgctccggcctg

SEQ ID NO: 11 - DNA, 29 bp, synthetic construct
  source 1..29: mol_type = other DNA
gggaagcttgacgtcggcccgccggcgcc

SEQ ID NO: 12 - DNA, 29 bp, synthetic construct
  source 1..29: mol_type = other DNA
cccaagcttgatttcttgatgttcctatg

SEQ ID NO: 13 - DNA, 29 bp, synthetic construct
  source 1..29: mol_type = other DNA
gggaagcttagttttcctcagctttgggt

SEQ ID NO: 14 - DNA, 27 bp, synthetic construct
  source 1..27: mol_type = other DNA
cccccatggcagggccgctcgctgggc

SEQ ID NO: 15 - DNA, 29 bp, synthetic construct
  source 1..29: mol_type = other DNA
gggaagcttacatttgcttctgacacaac

SEQ ID NO: 16 - DNA, 29 bp, synthetic construct
  source 1..29: mol_type = other DNA
cccccatgggtctgtttgaggttgctagt

SEQ ID NO: 17 - DNA, 26 bp, synthetic construct
  source 1..26: mol_type = other DNA
gggaagcttgaataaactagtatctc

SEQ ID NO: 18 - DNA, 25 bp, synthetic construct
  source 1..25: mol_type = other DNA
cccccatggggtggcgggttctctc

SEQ ID NO: 19 - DNA, 29 bp, synthetic construct
  source 1..29: mol_type = other DNA
gggaagcttagagactctccgaggcggcg

SEQ ID NO: 20 - DNA, 29 bp, synthetic construct
  source 1..29: mol_type = other DNA
cccccatggtttcccttaatttcgcttgc

SEQ ID NO: 21 - DNA, 59 bp, synthetic construct
  source 1..59: mol_type = other DNA
gggaagctttagatccttttaaattaaaaatgaagttttaaatcaatctaaagtatata

SEQ ID NO: 22 - DNA, 59 bp, synthetic construct
  source 1..59: mol_type = other DNA
cccccatggtatatactttagattgatttaaaacttcatttttaatttaaaaggatcta

SEQ ID NO: 23 - DNA, 377 bp, synthetic construct
  source 1..377: mol_type = other DNA
ctgtattgtctgaacttgcattgtgattggcctgtagagttgctgagagggctcgaggggtgggctggtatctcagaaagtgcctgacacactaaccaagctgagtttcctatgggaacaattgaagtaaactttttgttctggtcctttttggtcgaggagtaacaatacaaatggattttgggagtgactcaagaagtgaagaatgcacaagaatggatcacaagatggaatttatcaaaccctagccttgcttgttaaatttttttttttttttttttaagaatatctgtaatggtactgactttgcttgctttgaagtagctctttttttttttttttttttttttttgcagtaactgttttttaagtctctc

SEQ ID NO: 24 - DNA, 296 bp, synthetic construct
  source 1..296: mol_type = other DNA
gtaactgttttttaagtctctcgtagtgttaagttatagtgaatactgctacagcaatttctaatttttaagaattgagtaatggtgtagaacactaattcataatcactctaattaattgtaatctgaataaagtgtaacaattgtgtagcctttttgtataaaatagacaaatagaaaatggtccaattagtttcctttttaatatgcttaaaataagcaggtggatctatttcatgtttttgatcaaaaactatttgggatatgtatgggtagggtaaatcagtaagaggtgt

SEQ ID NO: 25 - DNA, 673 bp, synthetic construct
  source 1..673: mol_type = other DNA
ctgtattgtctgaacttgcattgtgattggcctgtagagttgctgagagggctcgaggggtgggctggtatctcagaaagtgcctgacacactaaccaagctgagtttcctatgggaacaattgaagtaaactttttgttctggtcctttttggtcgaggagtaacaatacaaatggattttgggagtgactcaagaagtgaagaatgcacaagaatggatcacaagatggaatttatcaaaccctagccttgcttgttaaatttttttttttttttttttaagaatatctgtaatggtactgactttgcttgctttgaagtagctctttttttttttttttttttttttttgcagtaactgttttttaagtctctcgtaactgttttttaagtctctcgtagtgttaagttatagtgaatactgctacagcaatttctaatttttaagaattgagtaatggtgtagaacactaattcataatcactctaattaattgtaatctgaataaagtgtaacaattgtgtagcctttttgtataaaatagacaaatagaaaatggtccaattagtttcctttttaatatgcttaaaataagcaggtggatctatttcatgtttttgatcaaaaactatttgggatatgtatgggtagggtaaatcagtaagaggtgt

SEQ ID NO: 26 - DNA, 36 bp, synthetic construct
  source 1..36: mol_type = other DNA
cgtgtaattctagactgtattgtctgaacttgcatt

SEQ ID NO: 27 - DNA, 90 bp, synthetic construct
  source 1..90: mol_type = other DNA
catcggtcgacggatccttttttttttttttttttttttttttttttttttttttttttttttttttttttttttttgagagacttaaaa

SEQ ID NO: 28 - DNA, 38 bp, synthetic construct
  source 1..38: mol_type = other DNA
cgtgtaattctagagtaactgttttttaagtctctcgt

SEQ ID NO: 29 - DNA, 90 bp, synthetic construct
  source 1..90: mol_type = other DNA
catcggtcgacggatccttttttttttttttttttttttttttttttttttttttttttttttttttttttttttttacacctcttactg

SEQ ID NO: 30 - DNA, 209 bp, synthetic construct
  source 1..209: mol_type = other DNA
ctgtttctctgcagttttcctcagctttgggtggtggccgctgccgggcatcggcttccagtccgcggagggcgaggcggcgtggacagcggccccggcacccagcgccccgccgcccgcaagccgcgcgcccgtccgccgcgccccgagcccgccgcttcctatctcagcgccctgccgccgccgccgcggcccagcgagcggccctg

SEQ ID NO: 31 - DNA, 54 bp, synthetic construct
  source 1..54: mol_type = other DNA
agttttcctcagctttgggtggtggccgctgccgggcatcggcttccagtccgc

SEQ ID NO: 32 - DNA, 71 bp, synthetic construct
  source 1..71: mol_type = other DNA
ggagggcgaggcggcgtggacagcggccccggcacccagcgccccgccgcccgcaagccgcgcgcccgtcc

SEQ ID NO: 33 - DNA, 72 bp, synthetic construct
  source 1..72: mol_type = other DNA
gccgcgccccgagcccgccgcttcctatctcagcgccctgccgccgccgccgcggcccagcgagcggccctg

SEQ ID NO: 34 - DNA, 125 bp, synthetic construct
  source 1..125: mol_type = other DNA
agttttcctcagctttgggtggtggccgctgccgggcatcggcttccagtccgcggagggcgaggcggcgtggacagcggccccggcacccagcgccccgccgcccgcaagccgcgcgcccgtcc

SEQ ID NO: 35 - DNA, 143 bp, synthetic construct
  source 1..143: mol_type = other DNA
ggagggcgaggcggcgtggacagcggccccggcacccagcgccccgccgcccgcaagccgcgcgcccgtccgccgcgccccgagcccgccgcttcctatctcagcgccctgccgccgccgccgcggcccagcgagcggccctg

SEQ ID NO: 36 - DNA, 126 bp, synthetic construct
  source 1..126: mol_type = other DNA
agttttcctcagctttgggtggtggccgctgccgggcatcggcttccagtccgcgccgcgccccgagcccgccgcttcctatctcagcgccctgccgccgccgccgcggcccagcgagcggccctg

SEQ ID NO: 37 - DNA, 29 bp, synthetic construct
  source 1..29: mol_type = other DNA
gggaagcttagttttcctcagctttgggt

SEQ ID NO: 38 - DNA, 40 bp, synthetic construct
  source 1..40: mol_type = other DNA
tgtttttggcgtcttccatgggcggactggaagccgatgc

SEQ ID NO: 39 - DNA, 23 bp, synthetic construct
  source 1..23: mol_type = other DNA
gggaagcttggagggcgaggcgg

SEQ ID NO: 40 - DNA, 35 bp, synthetic construct
  source 1..35: mol_type = other DNA
tgtttttggcgtcttccatggggacgggcgcgcgg

SEQ ID NO: 41 - DNA, 24 bp, synthetic construct
  source 1..24: mol_type = other DNA
gggaagcttgccgcgccccgagcc

SEQ ID NO: 42 - DNA, 38 bp, synthetic construct
  source 1..38: mol_type = other DNA
tgtttttggcgtcttccatggcagggccgctcgctggg

SEQ ID NO: 43 - DNA, 600 bp, synthetic construct
  source 1..600: mol_type = other DNA
gcggactatgacttagttgcgttacaccctttcttgacaaaacctaacttgcgcagaaaacaagatgagattggcatggctttatttgttttttttgttttgttttggttttttttttttttttggcttgactcaggatttaaaaactggaacggtgaaggtgacagcagtcggttggagcgagcatcccccaaagttcacaatgtggccgaggactttgattgcacattgttgtttttttaatagtcattccaaatatgagatgcgttgttacaggaagtcccttgccatcctaaaagccaccccacttctctctaaggagaatggcccagtcctctcccaagtccacacaggggaggtgatagcattgctttcgtgtaaattatgtaatgcaaaatttttttaatcttcgccttaatacttttttattttgttttattttgaatgatgagccttcgtgcccccccttcccccttttttgtcccccaacttgagatgtatgaaggcttttggtctccctgggagtgggtggaggcagccagggcttacctgtacactgacttgagaccagttgaataaaagtgcacaccttaaaaatga

SEQ ID NO: 44 - DNA, 268 bp, synthetic construct
  source 1..268: mol_type = other DNA
aggatacagcggcttctgcgcgacttataagagctccttgtgcggcgccattttaagcctctcggtctgtggcagcagcgttggcccggccccgggagcggagagcgaggggaggcggagacggaggaaggtctgaggagcagcttcagtccccgccgagccgccaccgcaggtcgaggacggtcggactcccgcggcgggaggagcctgttcccctgagggtatttgaagtataccatacaactgttttgaaaatccagcgtggaca

SEQ ID NO: 45 - DNA, 132 bp, synthetic construct
  source 1..132: mol_type = other DNA
gctcgctttcttgctgtccaatttctattaaaggttcctttgttccctaagtccaactactaaactgggggatattatgaagggccttgagcatctggattctgcctaataaaaaacatttattttcattgc

SEQ ID NO: 46 - DNA, 30 bp, synthetic construct
  source 1..30: mol_type = other DNA
cccggatccgcggactatgacttagttgcg

SEQ ID NO: 47 - DNA, 40 bp, synthetic construct
  source 1..40: mol_type = other DNA
ggggtcgactcatttttaaggtgtgcacttttattcaact

SEQ ID NO: 48 - DNA, 28 bp, synthetic construct
  source 1..28: mol_type = other DNA
cccggatccaggatacagcggcttctgc

SEQ ID NO: 49 - DNA, 33 bp, synthetic construct
  source 1..33: mol_type = other DNA
ggggtcgactgtccacgctggattttcaaaaca

SEQ ID NO: 50 - DNA, 27 bp, synthetic construct
  source 1..27: mol_type = other DNA
cccggatccgctcgctttcttgctgtc

SEQ ID NO: 51 - DNA, 29 bp, synthetic construct
  source 1..29: mol_type = other DNA
cccgctgacgcaatgaaaataaatgtttt

SEQ ID NO: 52 - DNA, 197 bp, synthetic construct
  source 1..197: mol_type = other DNA
agttttcctcagctttgggtggtggccgctgccgggcatcggcttccagtccgcggagggcgaggcagcgtggacagcggccccggcacccagcgccccgccgcccgcaagccgcgcgcccgtccgccgcgccccgagcccgccgcttcctatctcagcgccctgccgccgccgccgcggcccagcgagcggccctg

SEQ ID NO: 53 - DNA, 197 bp, synthetic construct
  source 1..197: mol_type = other DNA
agttttcctcagctttgggtggtggccgctgccgggcatcggcttccagtccgcggagggcgaggcagcgtagacagcggccccggcacccagcgccccgccgcccgcaagccgcgcgcccgtccgccgcgccccgagcccgccgcttcctatctcagcgccctgccgccgccgccgcggcccagcgagcggccctg

SEQ ID NO: 54 - DNA, 197 bp, synthetic construct
  source 1..197: mol_type = other DNA
agttttcctcagctttgggtggtggccgctgccgggcatcggcttccagtccgcggagggcgaggcagcgtagacagcagccccggcacccagcgccccgccgcccgcaagccgcgcgcccgtccgccgcgccccgagcccgccgcttcctatctcagcgccctgccgccgccgccgcggcccagcgagcggccctg

SEQ ID NO: 55 - DNA, 20 bp, synthetic construct
  source 1..20: mol_type = other DNA
agcgtggacagcggccccgg

SEQ ID NO: 56 - DNA, 20 bp, synthetic construct
  source 1..20: mol_type = other DNA
ccggggccgctgtccacgct

SEQ ID NO: 57 - DNA, 20 bp, synthetic construct
  source 1..20: mol_type = other DNA
agcgtagacagcggccccgg

SEQ ID NO: 58 - DNA, 20 bp, synthetic construct
  source 1..20: mol_type = other DNA
ccggggccgctgtctacgct

SEQ ID NO: 59 - DNA, 20 bp, synthetic construct
  source 1..20: mol_type = other DNA
agcgtagacagcagccccgg

SEQ ID NO: 60 - DNA, 20 bp, synthetic construct
  source 1..20: mol_type = other DNA
ccggggctgctgtctacgct

SEQ ID NO: 61 - DNA, 71 bp, synthetic construct
  source 1..71: mol_type = other DNA
ggagggcgaggcagcgtggacagcggccccggcacccagcgccccgccgcccgcaagccgcgcgcccgtcc

SEQ ID NO: 62 - DNA, 71 bp, synthetic construct
  source 1..71: mol_type = other DNA
ggagggcgaggcagcgtagacagcggccccggcacccagcgccccgccgcccgcaagccgcgcgcccgtcc

SEQ ID NO: 63 - DNA, 71 bp, synthetic construct
  source 1..71: mol_type = other DNA
ggagggcgaggcagcgtagacagcagccccggcacccagcgccccgccgcccgcaagccgcgcgcccgtcc

SEQ ID NO: 64 - DNA, 125 bp, synthetic construct
  source 1..125: mol_type = other DNA
agttttcctcagctttgggtggtggccgctgccgggcatcggcttccagtccgcggagggcgaggcagcgtggacagcggccccggcacccagcgccccgccgcccgcaagccgcgcgcccgtcc

SEQ ID NO: 65 - DNA, 125 bp, synthetic construct
  source 1..125: mol_type = other DNA
agttttcctcagctttgggtggtggccgctgccgggcatcggcttccagtccgcggagggcgaggcagcgtagacagcggccccggcacccagcgccccgccgcccgcaagccgcgcgcccgtcc

SEQ ID NO: 66 - DNA, 125 bp, synthetic construct
  source 1..125: mol_type = other DNA
agttttcctcagctttgggtggtggccgctgccgggcatcggcttccagtccgcggagggcgaggcagcgtagacagcagccccggcacccagcgccccgccgcccgcaagccgcgcgcccgtcc

SEQ ID NO: 67 - DNA, 143 bp, synthetic construct
  source 1..143: mol_type = other DNA
ggagggcgaggcagcgtggacagcggccccggcacccagcgccccgccgcccgcaagccgcgcgcccgtccgccgcgccccgagcccgccgcttcctatctcagcgccctgccgccgccgccgcggcccagcgagcggccctg

SEQ ID NO: 68 - DNA, 143 bp, synthetic construct
  source 1..143: mol_type = other DNA
ggagggcgaggcagcgtagacagcggccccggcacccagcgccccgccgcccgcaagccgcgcgcccgtccgccgcgccccgagcccgccgcttcctatctcagcgccctgccgccgccgccgcggcccagcgagcggccctg

SEQ ID NO: 69 - DNA, 143 bp, synthetic construct
  source 1..143: mol_type = other DNA
ggagggcgaggcagcgtagacagcagccccggcacccagcgccccgccgcccgcaagccgcgcgcccgtccgccgcgccccgagcccgccgcttcctatctcagcgccctgccgccgccgccgcggcccagcgagcggccctg